European Patent Specification EP 3 819 342 B1, published March 18, 2026. Title: Soft polyurethane foam, seat pad for automotive, and method for producing soft polyurethane foam. Applicant: Bridgestone Corporation Spiber Inc. The sequence listing filed with the application follows.

SEQUENCE LISTING (48 sequences)

SEQ ID NO: 1 - protein, 50 aa, Araneus diadematus
SGCDVLVQALLEVVSALVSILGSSSIGQINYGASAQYTQMVGQSVAQALA

SEQ ID NO: 2 - protein, 30 aa, Araneus diadematus
SGCDVLVQALLEVVSALVSILGSSSIGQIN

SEQ ID NO: 3 - protein, 21 aa, Araneus diadematus
SGCDVLVQALLEVVSALVSIL

SEQ ID NO: 4 - protein, 1154 aa, Artificial Sequence
  recombinant spider silk protein ADF3KaiLargeNRSH1
MHHHHHHHHHHSSGSSLEVLFQGPARAGSGQQGPGQQGPGQQGPGQQGPYGPGASAAAAAAGGYGPGSGQQGPSQQGPGQQGPGGQGPYGPGASAAAAAAGGYGPGSGQQGPGGQGPYGPGSSAAAAAAGGNGPGSGQQGAGQQGPGQQGPGASAAAAAAGGYGPGSGQQGPGQQGPGGQGPYGPGASAAAAAAGGYGPGSGQGPGQQGPGGQGPYGPGASAAAAAAGGYGPGSGQQGPGQQGPGQQGPGGQGPYGPGASAAAAAAGGYGPGYGQQGPGQQGPGGQGPYGPGASAASAASGGYGPGSGQQGPGQQGPGGQGPYGPGASAAAAAAGGYGPGSGQQGPGQQGPGQQGPGQQGPGGQGPYGPGASAAAAAAGGYGPGSGQQGPGQQGPGQQGPGQQGPGQQGPGQQGPGQQGPGQQGPGQQGPGGQGAYGPGASAAAGAAGGYGPGSGQQGPGQQGPGQQGPGQQGPGQQGPGQQGPGQQGPGQQGPYGPGASAAAAAAGGYGPGSGQQGPGQQGPGQQGPGGQGPYGPGAASAAVSVSRARAGSGQQGPGQQGPGQQGPGQQGPYGPGASAAAAAAGGYGPGSGQQGPSQQGPGQQGPGGQGPYGPGASAAAAAAGGYGPGSGQQGPGGQGPYGPGSSAAAAAAGGNGPGSGQQGAGQQGPGQQGPGASAAAAAAGGYGPGSGQQGPGQQGPGGQGPYGPGASAAAAAAGGYGPGSGQGPGQQGPGGQGPYGPGASAAAAAAGGYGPGSGQQGPGQQGPGQQGPGGQGPYGPGASAAAAAAGGYGPGYGQQGPGQQGPGGQGPYGPGASAASAASGGYGPGSGQQGPGQQGPGGQGPYGPGASAAAAAAGGYGPGSGQQGPGQQGPGQQGPGQQGPGGQGPYGPGASAAAAAAGGYGPGSGQQGPGQQGPGQQGPGQQGPGQQGPGQQGPGQQGPGQQGPGQQGPGGQGAYGPGASAAAGAAGGYGPGSGQQGPGQQGPGQQGPGQQGPGQQGPGQQGPGQQGPGQQGPYGPGASAAAAAAGGYGPGSGQQGPGQQGPGQQGPGGQGPYGPGAASAAVSVGGYGPQSSSVPVASAVASRLSSPAASSRVSSAVSSLVSSGPTKHAALSNTISSVVSQVSASNPGLSGCDVLVQALLEVVSALVSIL

SEQ ID NO: 5 - protein, 24 aa, Artificial Sequence
  His tag and start codon
MHHHHHHHHHHSSGSSLEVLFQGP

SEQ ID NO: 6 - protein, 597 aa, Artificial Sequence
  Met-PRT380
MGPGQQGPYGPGASAAAAAGQNGPGSGQQGPGQSAAAAAGQYGPGQQGPGQQGPGSSAAAAAGPGQYGPGQQGPSASAAAAAGPGSGQQGPGASAAAAAGQYGPGQQGPGQQGPGSSAAAAAGQYGSGPGQQGPYGSAAAAAGPGSGQYGQGPYGPGASAAAAAGPGQYGPGQQGPSASAAAAAGSGQQGPGQYGPYASAAAAAGQYGSGPGQQGPYGPGQSAAAAAGSGQQGPGQQGPYASAAAAAGPGQQGPYGPGSSAAAAAGQYGYGPGQQGPYGPGASAAAAAGQNGPGSGQYGPGQQGPGQSAAAAAGPGQQGPYGPGASAAAAAGQYGPGQQGPGQYGPGSSAAAAAGPGQQGPYGPGSSAAAAAGQYGPGQQGPYGPGQSAAAAAGQYQQGPGQQGPYGPGASAAAAAGPGQQGPYGPGASAAAAAGPGQYGPGQQGPSASAAAAAGQYGSGPGQYGPYGPGQSAAAAAGPGSGQQGQGPYGPGASAAAAAGQYGPGQQGPYGPGQSAAAAAGPGSGQYGPGASAAAAAGQNGPGSGQYGPGQQGPGQSAAAAAGQYQQGPGQQGPYGPGASAAAAAGPGSGQQGPGAS

SEQ ID NO: 7 - protein, 590 aa, Artificial Sequence
  Met-PRT410
MGPGQQGPYGPGASAAAAAGQNGPGSGQQGPGQSGQYGPGQQGPGQQGPGSSAAAAAGPGQYGPGQQGPSASAAAAAGPGSGQQGPGASGQYGPGQQGPGQQGPGSSAAAAAGQYGSGPGQQGPYGSAAAAAGPGSGQYGQGPYGPGASGPGQYGPGQQGPSASAAAAAGSGQQGPGQYGPYASAAAAAGQYGSGPGQQGPYGPGQSGSGQQGPGQQGPYASAAAAAGPGQQGPYGPGSSAAAAAGQYGYGPGQQGPYGPGASGQNGPGSGQYGPGQQGPGQSAAAAAGPGQQGPYGPGASAAAAAGQYGPGQQGPGQYGPGSSGPGQQGPYGPGSSAAAAAGQYGPGQQGPYGPGQSAAAAAGQYQQGPGQQGPYGPGASGPGQQGPYGPGASAAAAAGPGQYGPGQQGPSASAAAAAGQYGSGPGQYGPYGPGQSGPGSGQQGQGPYGPGASAAAAAGQYGPGQQGPYGPGQSAAAAAGPGSGQYGPGASGQNGPGSGQYGPGQQGPGQSAAAAAGQYQQGPGQQGPYGPGASAAAAAGQYGSGPGQQGPYGPGQSGSGQQGPGQQGPYASAAAAAGPGSGQQGPGAS

SEQ ID NO: 8 - protein, 565 aa, Artificial Sequence
  Met-PRT525
MGPGQQGPYGPGASAAAAAAAGSNGPGSGQQGPGQSGQYGPGQQGPGQQGPGSSAAAAAAAGPGQYGPGQQGPSASAAAAAAAGPGSGQQGPGASGQYGPGQQGPGQQGPGSSAAAAAAAGSYGSGPGQQGPYGSAAAAAAAGPGSGQYGQGPYGPGASGPGQYGPGQQGPSASAAAAAAAGSGQQGPGQYGPYASAAAAAAAGSYGSGPGQQGPYGPGQSGSGQQGPGQQGPYASAAAAAAAGPGQQGPYGPGSSAAAAAAAGSYGYGPGQQGPYGPGASGQNGPGSGQYGPGQQGPGPSAAAAAAAGPGQQGPYGPGASAAAAAAAGSYGPGQQGPGQYGPGSSGPGQQGPYGPGSSAAAAAAAGSYGPGQQGPYGPGPSAAAAAAAGSYQQGPGQQGPYGPGASGPGQQGPYGPGASAAAAAAAGPGQYGPGQQGPSASAAAAAAAGSYGSGPGQYGPYGPGQSGPGSGQQGQGPYGPGASAAAAAAAGSYGPGQQGPYGPGPSAAAAAAAGPGSGQYGPGASGQNGPGSGQYGPGQQGPGPSAAAAAAAGPGSGQQGPGAS

SEQ ID NO: 9 - protein, 2364 aa, Artificial Sequence
  Met-PRT799
MGPGQQGPYGPGASAAAAAGQNGPGSGQQGPGQSGQYGPGQQGPGQQGPGSSAAAAAGPGQYGPGQQGPSASAAAAAGPGSGQQGPGASGQYGPGQQGPGQQGPGSSAAAAAGQYGSGPGQQGPYGSAAAAAGPGSGQYGQGPYGPGASGPGQYGPGQQGPSASAAAAAGSGQQGPGQYGPYASAAAAAGQYGSGPGQQGPYGPGQSGSGQQGPGQQGPYASAAAAAGPGQQGPYGPGSSAAAAAGQYGYGPGQQGPYGPGASGQNGPGSGQYGPGQQGPGQSAAAAAGPGQQGPYGPGASAAAAAGQYGPGQQGPGQYGPGSSGPGQQGPYGPGSSAAAAAGQYGPGQQGPYGPGQSAAAAAGQYQQGPGQQGPYGPGASGPGQQGPYGPGASAAAAAGPGQYGPGQQGPSASAAAAAGQYGSGPGQYGPYGPGQSGPGSGQQGQGPYGPGASAAAAAGQYGPGQQGPYGPGQSAAAAAGPGSGQYGPGASGQNGPGSGQYGPGQQGPGQSAAAAAGQYQQGPGQQGPYGPGASAAAAAGQYGSGPGQQGPYGPGQSGSGQQGPGQQGPYASAAAAAGPGSGQQGPGASGQQGPYGPGASAAAAAGQNGPGSGQQGPGQSGQYGPGQQGPGQQGPGSSAAAAAGPGQYGPGQQGPSASAAAAAGPGSGQQGPGASGQYGPGQQGPGQQGPGSSAAAAAGQYGSGPGQQGPYGSAAAAAGPGSGQYGQGPYGPGASGPGQYGPGQQGPSASAAAAAGSGQQGPGQYGPYASAAAAAGQYGSGPGQQGPYGPGQSGSGQQGPGQQGPYASAAAAAGPGQQGPYGPGSSAAAAAGQYGYGPGQQGPYGPGASGQNGPGSGQYGPGQQGPGQSAAAAAGPGQQGPYGPGASAAAAAGQYGPGQQGPGQYGPGSSGPGQQGPYGPGSSAAAAAGQYGPGQQGPYGPGQSAAAAAGQYQQGPGQQGPYGPGASGPGQQGPYGPGASAAAAAGPGQYGPGQQGPSASAAAAAGQYGSGPGQYGPYGPGQSGPGSGQQGQGPYGPGASAAAAAGQYGPGQQGPYGPGQSAAAAAGPGSGQYGPGASGQNGPGSGQYGPGQQGPGQSAAAAAGQYQQGPGQQGPYGPGASAAAAAGQYGSGPGQQGPYGPGQSGSGQQGPGQQGPYASAAAAAGPGSGQQGPGASGQQGPYGPGASAAAAAGQNGPGSGQQGPGQSGQYGPGQQGPGQQGPGSSAAAAAGPGQYGPGQQGPSASAAAAAGPGSGQQGPGASGQYGPGQQGPGQQGPGSSAAAAAGQYGSGPGQQGPYGSAAAAAGPGSGQYGQGPYGPGASGPGQYGPGQQGPSASAAAAAGSGQQGPGQYGPYASAAAAAGQYGSGPGQQGPYGPGQSGSGQQGPGQQGPYASAAAAAGPGQQGPYGPGSSAAAAAGQYGYGPGQQGPYGPGASGQNGPGSGQYGPGQQGPGQSAAAAAGPGQQGPYGPGASAAAAAGQYGPGQQGPGQYGPGSSGPGQQGPYGPGSSAAAAAGQYGPGQQGPYGPGQSAAAAAGQYQQGPGQQGPYGPGASGPGQQGPYGPGASAAAAAGPGQYGPGQQGPSASAAAAAGQYGSGPGQYGPYGPGQSGPGSGQQGQGPYGPGASAAAAAGQYGPGQQGPYGPGQSAAAAAGPGSGQYGPGASGQNGPGSGQYGPGQQGPGQSAAAAAGQYQQGPGQQGPYGPGASAAAAAGQYGSGPGQQGPYGPGQSGSGQQGPGQQGPYASAAAAAGPGSGQQGPGASGQQGPYGPGASAAAAAGQNGPGSGQQGPGQSGQYGPGQQGPGQQGPGSSAAAAAGPGQYGPGQQGPSASAAAAAGPGSGQQGPGASGQYGPGQQGPGQQGPGSSAAAAAGQYGSGPGQQGPYGSAAAAAGPGSGQYGQGPYGPGASGPGQYGPGQQGPSASAAAAAGSGQQGPGQYGPYASAAAAAGQYGSGPGQQGPYGPGQSGSGQQGPGQQGPYASAAAAAGPGQQGPYGPGSSAAAAAGQYGYGPGQQGPYGPGASGQNGPGSGQYGPGQQGPGQSAAAAAGPGQQGPYGPGASAAAAAGQYGPGQQGPGQYGPGSSGPGQQGPYGPGSSAAAAAGQYGPGQQGPYGPGQSAAAAAGQYQQGPGQQGPYGPGASGPGQQGPYGPGASAAAAAGPGQYGPGQQGPSASAAAAAGQYGSGPGQYGPYGPGQSGPGSGQQGQGPYGPGASAAAAAGQYGPGQQGPYGPGQSAAAAAGPGSGQYGPGASGQNGPGSGQYGPGQQGPGQSAAAAAGQYQQGPGQQGPYGPGASAAAAAGQYGSGPGQQGPYGPGQSGSGQQGPGQQGPYASAAAAAGPGSGQQGSSVDKLAAALEHHHHHH

SEQ ID NO: 10 - protein, 597 aa, Artificial Sequence
  Met-PRT313
MGPGGQGPYGPGASAAAAAGGNGPGSGQQGPGGSAAAAAGGYGPGGQGPGQQGPGSSAAAAAGPGGYGPGGQGPSASAAAAAGPGSGQQGPGASAAAAAGGYGPGGQGPGQQGPGSSAAAAAGGYGSGPGQQGPYGSAAAAAGPGSGGYGQGPYGPGASAAAAAGPGGYGPGGQGPSASAAAAAGSGQQGPGGYGPYASAAAAAGGYGSGPGQQGPYGPGGSAAAAAGSGQQGPGQQGPYASAAAAAGPGGQGPYGPGSSAAAAAGGYGYGPGGQGPYGPGASAAAAAGGNGPGSGGYGPGQQGPGGSAAAAAGPGGQGPYGPGASAAAAAGGYGPGGQGPGGYGPGSSAAAAAGPGGQGPYGPGSSAAAAAGGYGPGQQGPYGPGGSAAAAAGGYQQGPGGQGPYGPGASAAAAAGPGGQGPYGPGASAAAAAGPGGYGPGGQGPSASAAAAAGGYGSGPGGYGPYGPGGSAAAAAGPGSGQQGQGPYGPGASAAAAAGGYGPGQQGPYGPGGSAAAAAGPGSGGYGPGASAAAAAGGNGPGSGGYGPGQQGPGGSAAAAAGGYQQGPGGQGPYGPGASAAAAAGPGSGQQGPGAS

SEQ ID NO: 11 - protein, 12 aa, Artificial Sequence
  HisTag
MHHHHHHSSGSS

SEQ ID NO: 12 - protein, 608 aa, Artificial Sequence
  PRT380
MHHHHHHSSGSSGPGQQGPYGPGASAAAAAGQNGPGSGQQGPGQSAAAAAGQYGPGQQGPGQQGPGSSAAAAAGPGQYGPGQQGPSASAAAAAGPGSGQQGPGASAAAAAGQYGPGQQGPGQQGPGSSAAAAAGQYGSGPGQQGPYGSAAAAAGPGSGQYGQGPYGPGASAAAAAGPGQYGPGQQGPSASAAAAAGSGQQGPGQYGPYASAAAAAGQYGSGPGQQGPYGPGQSAAAAAGSGQQGPGQQGPYASAAAAAGPGQQGPYGPGSSAAAAAGQYGYGPGQQGPYGPGASAAAAAGQNGPGSGQYGPGQQGPGQSAAAAAGPGQQGPYGPGASAAAAAGQYGPGQQGPGQYGPGSSAAAAAGPGQQGPYGPGSSAAAAAGQYGPGQQGPYGPGQSAAAAAGQYQQGPGQQGPYGPGASAAAAAGPGQQGPYGPGASAAAAAGPGQYGPGQQGPSASAAAAAGQYGSGPGQYGPYGPGQSAAAAAGPGSGQQGQGPYGPGASAAAAAGQYGPGQQGPYGPGQSAAAAAGPGSGQYGPGASAAAAAGQNGPGSGQYGPGQQGPGQSAAAAAGQYQQGPGQQGPYGPGASAAAAAGPGSGQQGPGAS

SEQ ID NO: 13 - protein, 601 aa, Artificial Sequence
  PRT410
MHHHHHHSSGSSGPGQQGPYGPGASAAAAAGQNGPGSGQQGPGQSGQYGPGQQGPGQQGPGSSAAAAAGPGQYGPGQQGPSASAAAAAGPGSGQQGPGASGQYGPGQQGPGQQGPGSSAAAAAGQYGSGPGQQGPYGSAAAAAGPGSGQYGQGPYGPGASGPGQYGPGQQGPSASAAAAAGSGQQGPGQYGPYASAAAAAGQYGSGPGQQGPYGPGQSGSGQQGPGQQGPYASAAAAAGPGQQGPYGPGSSAAAAAGQYGYGPGQQGPYGPGASGQNGPGSGQYGPGQQGPGQSAAAAAGPGQQGPYGPGASAAAAAGQYGPGQQGPGQYGPGSSGPGQQGPYGPGSSAAAAAGQYGPGQQGPYGPGQSAAAAAGQYQQGPGQQGPYGPGASGPGQQGPYGPGASAAAAAGPGQYGPGQQGPSASAAAAAGQYGSGPGQYGPYGPGQSGPGSGQQGQGPYGPGASAAAAAGQYGPGQQGPYGPGQSAAAAAGPGSGQYGPGASGQNGPGSGQYGPGQQGPGQSAAAAAGQYQQGPGQQGPYGPGASAAAAAGQYGSGPGQQGPYGPGQSGSGQQGPGQQGPYASAAAAAGPGSGQQGPGAS

SEQ ID NO: 14 - protein, 576 aa, Artificial Sequence
  PRT525
MHHHHHHSSGSSGPGQQGPYGPGASAAAAAAAGSNGPGSGQQGPGQSGQYGPGQQGPGQQGPGSSAAAAAAAGPGQYGPGQQGPSASAAAAAAAGPGSGQQGPGASGQYGPGQQGPGQQGPGSSAAAAAAAGSYGSGPGQQGPYGSAAAAAAAGPGSGQYGQGPYGPGASGPGQYGPGQQGPSASAAAAAAAGSGQQGPGQYGPYASAAAAAAAGSYGSGPGQQGPYGPGQSGSGQQGPGQQGPYASAAAAAAAGPGQQGPYGPGSSAAAAAAAGSYGYGPGQQGPYGPGASGQNGPGSGQYGPGQQGPGPSAAAAAAAGPGQQGPYGPGASAAAAAAAGSYGPGQQGPGQYGPGSSGPGQQGPYGPGSSAAAAAAAGSYGPGQQGPYGPGPSAAAAAAAGSYQQGPGQQGPYGPGASGPGQQGPYGPGASAAAAAAAGPGQYGPGQQGPSASAAAAAAAGSYGSGPGQYGPYGPGQSGPGSGQQGQGPYGPGASAAAAAAAGSYGPGQQGPYGPGPSAAAAAAAGPGSGQYGPGASGQNGPGSGQYGPGQQGPGPSAAAAAAAGPGSGQQGPGAS

SEQ ID NO: 15 - protein, 2375 aa, Artificial Sequence
  PRT799
MHHHHHHSSGSSGPGQQGPYGPGASAAAAAGQNGPGSGQQGPGQSGQYGPGQQGPGQQGPGSSAAAAAGPGQYGPGQQGPSASAAAAAGPGSGQQGPGASGQYGPGQQGPGQQGPGSSAAAAAGQYGSGPGQQGPYGSAAAAAGPGSGQYGQGPYGPGASGPGQYGPGQQGPSASAAAAAGSGQQGPGQYGPYASAAAAAGQYGSGPGQQGPYGPGQSGSGQQGPGQQGPYASAAAAAGPGQQGPYGPGSSAAAAAGQYGYGPGQQGPYGPGASGQNGPGSGQYGPGQQGPGQSAAAAAGPGQQGPYGPGASAAAAAGQYGPGQQGPGQYGPGSSGPGQQGPYGPGSSAAAAAGQYGPGQQGPYGPGQSAAAAAGQYQQGPGQQGPYGPGASGPGQQGPYGPGASAAAAAGPGQYGPGQQGPSASAAAAAGQYGSGPGQYGPYGPGQSGPGSGQQGQGPYGPGASAAAAAGQYGPGQQGPYGPGQSAAAAAGPGSGQYGPGASGQNGPGSGQYGPGQQGPGQSAAAAAGQYQQGPGQQGPYGPGASAAAAAGQYGSGPGQQGPYGPGQSGSGQQGPGQQGPYASAAAAAGPGSGQQGPGASGQQGPYGPGASAAAAAGQNGPGSGQQGPGQSGQYGPGQQGPGQQGPGSSAAAAAGPGQYGPGQQGPSASAAAAAGPGSGQQGPGASGQYGPGQQGPGQQGPGSSAAAAAGQYGSGPGQQGPYGSAAAAAGPGSGQYGQGPYGPGASGPGQYGPGQQGPSASAAAAAGSGQQGPGQYGPYASAAAAAGQYGSGPGQQGPYGPGQSGSGQQGPGQQGPYASAAAAAGPGQQGPYGPGSSAAAAAGQYGYGPGQQGPYGPGASGQNGPGSGQYGPGQQGPGQSAAAAAGPGQQGPYGPGASAAAAAGQYGPGQQGPGQYGPGSSGPGQQGPYGPGSSAAAAAGQYGPGQQGPYGPGQSAAAAAGQYQQGPGQQGPYGPGASGPGQQGPYGPGASAAAAAGPGQYGPGQQGPSASAAAAAGQYGSGPGQYGPYGPGQSGPGSGQQGQGPYGPGASAAAAAGQYGPGQQGPYGPGQSAAAAAGPGSGQYGPGASGQNGPGSGQYGPGQQGPGQSAAAAAGQYQQGPGQQGPYGPGASAAAAAGQYGSGPGQQGPYGPGQSGSGQQGPGQQGPYASAAAAAGPGSGQQGPGASGQQGPYGPGASAAAAAGQNGPGSGQQGPGQSGQYGPGQQGPGQQGPGSSAAAAAGPGQYGPGQQGPSASAAAAAGPGSGQQGPGASGQYGPGQQGPGQQGPGSSAAAAAGQYGSGPGQQGPYGSAAAAAGPGSGQYGQGPYGPGASGPGQYGPGQQGPSASAAAAAGSGQQGPGQYGPYASAAAAAGQYGSGPGQQGPYGPGQSGSGQQGPGQQGPYASAAAAAGPGQQGPYGPGSSAAAAAGQYGYGPGQQGPYGPGASGQNGPGSGQYGPGQQGPGQSAAAAAGPGQQGPYGPGASAAAAAGQYGPGQQGPGQYGPGSSGPGQQGPYGPGSSAAAAAGQYGPGQQGPYGPGQSAAAAAGQYQQGPGQQGPYGPGASGPGQQGPYGPGASAAAAAGPGQYGPGQQGPSASAAAAAGQYGSGPGQYGPYGPGQSGPGSGQQGQGPYGPGASAAAAAGQYGPGQQGPYGPGQSAAAAAGPGSGQYGPGASGQNGPGSGQYGPGQQGPGQSAAAAAGQYQQGPGQQGPYGPGASAAAAAGQYGSGPGQQGPYGPGQSGSGQQGPGQQGPYASAAAAAGPGSGQQGPGASGQQGPYGPGASAAAAAGQNGPGSGQQGPGQSGQYGPGQQGPGQQGPGSSAAAAAGPGQYGPGQQGPSASAAAAAGPGSGQQGPGASGQYGPGQQGPGQQGPGSSAAAAAGQYGSGPGQQGPYGSAAAAAGPGSGQYGQGPYGPGASGPGQYGPGQQGPSASAAAAAGSGQQGPGQYGPYASAAAAAGQYGSGPGQQGPYGPGQSGSGQQGPGQQGPYASAAAAAGPGQQGPYGPGSSAAAAAGQYGYGPGQQGPYGPGASGQNGPGSGQYGPGQQGPGQSAAAAAGPGQQGPYGPGASAAAAAGQYGPGQQGPGQYGPGSSGPGQQGPYGPGSSAAAAAGQYGPGQQGPYGPGQSAAAAAGQYQQGPGQQGPYGPGASGPGQQGPYGPGASAAAAAGPGQYGPGQQGPSASAAAAAGQYGSGPGQYGPYGPGQSGPGSGQQGQGPYGPGASAAAAAGQYGPGQQGPYGPGQSAAAAAGPGSGQYGPGASGQNGPGSGQYGPGQQGPGQSAAAAAGQYQQGPGQQGPYGPGASAAAAAGQYGSGPGQQGPYGPGQSGSGQQGPGQQGPYASAAAAAGPGSGQQGSSVDKLAAALEHHHHHH

SEQ ID NO: 16 - protein, 608 aa, Artificial Sequence
  PRT313
MHHHHHHSSGSSGPGGQGPYGPGASAAAAAGGNGPGSGQQGPGGSAAAAAGGYGPGGQGPGQQGPGSSAAAAAGPGGYGPGGQGPSASAAAAAGPGSGQQGPGASAAAAAGGYGPGGQGPGQQGPGSSAAAAAGGYGSGPGQQGPYGSAAAAAGPGSGGYGQGPYGPGASAAAAAGPGGYGPGGQGPSASAAAAAGSGQQGPGGYGPYASAAAAAGGYGSGPGQQGPYGPGGSAAAAAGSGQQGPGQQGPYASAAAAAGPGGQGPYGPGSSAAAAAGGYGYGPGGQGPYGPGASAAAAAGGNGPGSGGYGPGQQGPGGSAAAAAGPGGQGPYGPGASAAAAAGGYGPGGQGPGGYGPGSSAAAAAGPGGQGPYGPGSSAAAAAGGYGPGQQGPYGPGGSAAAAAGGYQQGPGGQGPYGPGASAAAAAGPGGQGPYGPGASAAAAAGPGGYGPGGQGPSASAAAAAGGYGSGPGGYGPYGPGGSAAAAAGPGSGQQGQGPYGPGASAAAAAGGYGPGQQGPYGPGGSAAAAAGPGSGGYGPGASAAAAAGGNGPGSGGYGPGQQGPGGSAAAAAGGYQQGPGGQGPYGPGASAAAAAGPGSGQQGPGAS

SEQ ID NO: 17 - protein, 590 aa, Artificial Sequence
  Met-PRT399
MGPGGQGPYGPGASAAAAAGGNGPGSGQQGPGGSGGYGPGGQGPGQQGPGSSAAAAAGPGGYGPGGQGPSASAAAAAGPGSGQQGPGASGGYGPGGQGPGQQGPGSSAAAAAGGYGSGPGQQGPYGSAAAAAGPGSGGYGQGPYGPGASGPGGYGPGGQGPSASAAAAAGSGQQGPGGYGPYASAAAAAGGYGSGPGQQGPYGPGGSGSGQQGPGQQGPYASAAAAAGPGGQGPYGPGSSAAAAAGGYGYGPGGQGPYGPGASGGNGPGSGGYGPGQQGPGGSAAAAAGPGGQGPYGPGASAAAAAGGYGPGGQGPGGYGPGSSGPGGQGPYGPGSSAAAAAGGYGPGQQGPYGPGGSAAAAAGGYQQGPGGQGPYGPGASGPGGQGPYGPGASAAAAAGPGGYGPGGQGPSASAAAAAGGYGSGPGGYGPYGPGGSGPGSGQQGQGPYGPGASAAAAAGGYGPGQQGPYGPGGSAAAAAGPGSGGYGPGASGGNGPGSGGYGPGQQGPGGSAAAAAGGYQQGPGGQGPYGPGASAAAAAGGYGSGPGQQGPYGPGGSGSGQQGPGQQGPYASAAAAAGPGSGQQGPGAS

SEQ ID NO: 18 - protein, 601 aa, Artificial Sequence
  PRT399
MHHHHHHSSGSSGPGGQGPYGPGASAAAAAGGNGPGSGQQGPGGSGGYGPGGQGPGQQGPGSSAAAAAGPGGYGPGGQGPSASAAAAAGPGSGQQGPGASGGYGPGGQGPGQQGPGSSAAAAAGGYGSGPGQQGPYGSAAAAAGPGSGGYGQGPYGPGASGPGGYGPGGQGPSASAAAAAGSGQQGPGGYGPYASAAAAAGGYGSGPGQQGPYGPGGSGSGQQGPGQQGPYASAAAAAGPGGQGPYGPGSSAAAAAGGYGYGPGGQGPYGPGASGGNGPGSGGYGPGQQGPGGSAAAAAGPGGQGPYGPGASAAAAAGGYGPGGQGPGGYGPGSSGPGGQGPYGPGSSAAAAAGGYGPGQQGPYGPGGSAAAAAGGYQQGPGGQGPYGPGASGPGGQGPYGPGASAAAAAGPGGYGPGGQGPSASAAAAAGGYGSGPGGYGPYGPGGSGPGSGQQGQGPYGPGASAAAAAGGYGPGQQGPYGPGGSAAAAAGPGSGGYGPGASGGNGPGSGGYGPGQQGPGGSAAAAAGGYQQGPGGQGPYGPGASAAAAAGGYGSGPGQQGPYGPGGSGSGQQGPGQQGPYASAAAAAGPGSGQQGPGAS

SEQ ID NO: 19 - protein, 612 aa, Artificial Sequence
  Met-PRT720
MGPGQQGPYGPGASAAAAAGQNGPGSGQQGPGQSGQYGPGQQGPGQQGPGSSAAAAAGPGQYVLIGPGQQVLIGPSASAAAAAGPGSGQQGPGASGQYGPGQQGPGQQGPGSSAAAAAGSYGSVLIGPGQQVLIGPYGSAAAAAGPGSGQYGQGPYGPGASGPGQYGPGQQGPSASAAAAAGSGQQVLIGPGQYVLIGPYASAAAAAGQYGSGPGQQGPYGPGQSGSGQQGPGQQGPYASAAAAAGPGQQVLIGPYVLIGPGSSAAAAAGQYGYGPGQQGPYGPGASGQNGPGSGQYGPGQQGPGQSAAAAAGPGQQVLIGPYVLIGPGASAAAAAGQYGPGQQGPGQYGPGSSGPGQQGPYGPGSSAAAAAGSYGPGQQVLIGPYVLIGPGPSAAAAAGQYQQGPGQQGPYGPGASGPGQQGPYGPGASAAAAAGPGQYVLIGPGQQVLIGPSASAAAAAGQYGSGPGQYGPYGPGQSGPGSGQQGQGPYGPGASAAAAAGSYGPGQQVLIGPYVLIGPGPSAAAAAGPGSGQYGPGASGQNGPGSGQYGPGQQGPGQSAAAAAGQYQQVLIGPGQQGPYVLIGPGASAAAAAGPGSGQQVLIGPGASVLI

SEQ ID NO: 20 - protein, 592 aa, Artificial Sequence
  Met-PRT665
MGPGQQGPYGPGASAAAAAAAGSNGPGSGQQGPGQSGQYGPGQQGPGQQGPGSSAAAAAAAGPGQYVLIGPGQQGPSASAAAAAAAGPGSGQQGPGASGQYGPGQQGPGQQGPGSSAAAAAAAGSYGSVLIGPGQQGPYGSAAAAAAAGPGSGQYGQGPYGPGASGPGQYGPGQQGPSASAAAAAAAGSGQQVLIGPGQYGPYASAAAAAAAGSYGSGPGQQGPYGPGQSGSGQQGPGQQGPYASAAAAAAAGPGQQVLIGPYGPGSSAAAAAAAGSYGYGPGQQGPYGPGASGQNGPGSGQYGPGQQGPGPSAAAAAAAGPGQQVLIGPYGPGASAAAAAAAGSYGPGQQGPGQYGPGSSGPGQQGPYGPGSSAAAAAAAGSYGPGQQVLIGPYGPGPSAAAAAAAGSYQQGPGQQGPYGPGASGPGQQGPYGPGASAAAAAAAGPGQYVLIGPGQQGPSASAAAAAAAGSYGSGPGQYGPYGPGQSGPGSGQQGQGPYGPGASAAAAAAAGSYGPGQQVLIGPYGPGPSAAAAAAAGPGSGQYGPGASGQNGPGSGQYGPGQQGPGPSAAAAAAAGPGSGQQGPGASVLI

SEQ ID NO: 21 - protein, 619 aa, Artificial Sequence
  Met-PRT666
MGPGQQGPYGPGASAAAAAAAGSNGPGSGQQGPGQSGQYGPGQQGPGQQGPGSSAAAAAAAGPGQYVLIGPGQQVLIGPSASAAAAAAAGPGSGQQGPGASGQYGPGQQGPGQQGPGSSAAAAAAAGSYGSVLIGPGQQVLIGPYGSAAAAAAAGPGSGQYGQGPYGPGASGPGQYGPGQQGPSASAAAAAAAGSGQQVLIGPGQYVLIGPYASAAAAAAAGSYGSGPGQQGPYGPGQSGSGQQGPGQQGPYASAAAAAAAGPGQQVLIGPYVLIGPGSSAAAAAAAGSYGYGPGQQGPYGPGASGQNGPGSGQYGPGQQGPGPSAAAAAAAGPGQQVLIGPYVLIGPGASAAAAAAAGSYGPGQQGPGQYGPGSSGPGQQGPYGPGSSAAAAAAAGSYGPGQQVLIGPYVLIGPGPSAAAAAAAGSYQQGPGQQGPYGPGASGPGQQGPYGPGASAAAAAAAGPGQYVLIGPGQQVLIGPSASAAAAAAAGSYGSGPGQYGPYGPGQSGPGSGQQGQGPYGPGASAAAAAAAGSYGPGQQVLIGPYVLIGPGPSAAAAAAAGPGSGQYGPGASGQNGPGSGQYGPGQQGPGPSAAAAAAAGPGSGQQVLIGPGASVLI

SEQ ID NO: 22 - protein, 623 aa, Artificial Sequence
  PRT720
MHHHHHHSSGSSGPGQQGPYGPGASAAAAAGQNGPGSGQQGPGQSGQYGPGQQGPGQQGPGSSAAAAAGPGQYVLIGPGQQVLIGPSASAAAAAGPGSGQQGPGASGQYGPGQQGPGQQGPGSSAAAAAGSYGSVLIGPGQQVLIGPYGSAAAAAGPGSGQYGQGPYGPGASGPGQYGPGQQGPSASAAAAAGSGQQVLIGPGQYVLIGPYASAAAAAGQYGSGPGQQGPYGPGQSGSGQQGPGQQGPYASAAAAAGPGQQVLIGPYVLIGPGSSAAAAAGQYGYGPGQQGPYGPGASGQNGPGSGQYGPGQQGPGQSAAAAAGPGQQVLIGPYVLIGPGASAAAAAGQYGPGQQGPGQYGPGSSGPGQQGPYGPGSSAAAAAGSYGPGQQVLIGPYVLIGPGPSAAAAAGQYQQGPGQQGPYGPGASGPGQQGPYGPGASAAAAAGPGQYVLIGPGQQVLIGPSASAAAAAGQYGSGPGQYGPYGPGQSGPGSGQQGQGPYGPGASAAAAAGSYGPGQQVLIGPYVLIGPGPSAAAAAGPGSGQYGPGASGQNGPGSGQYGPGQQGPGQSAAAAAGQYQQVLIGPGQQGPYVLIGPGASAAAAAGPGSGQQVLIGPGASVLI

SEQ ID NO: 23 - protein, 603 aa, Artificial Sequence
  PRT665
MHHHHHHSSGSSGPGQQGPYGPGASAAAAAAAGSNGPGSGQQGPGQSGQYGPGQQGPGQQGPGSSAAAAAAAGPGQYVLIGPGQQGPSASAAAAAAAGPGSGQQGPGASGQYGPGQQGPGQQGPGSSAAAAAAAGSYGSVLIGPGQQGPYGSAAAAAAAGPGSGQYGQGPYGPGASGPGQYGPGQQGPSASAAAAAAAGSGQQVLIGPGQYGPYASAAAAAAAGSYGSGPGQQGPYGPGQSGSGQQGPGQQGPYASAAAAAAAGPGQQVLIGPYGPGSSAAAAAAAGSYGYGPGQQGPYGPGASGQNGPGSGQYGPGQQGPGPSAAAAAAAGPGQQVLIGPYGPGASAAAAAAAGSYGPGQQGPGQYGPGSSGPGQQGPYGPGSSAAAAAAAGSYGPGQQVLIGPYGPGPSAAAAAAAGSYQQGPGQQGPYGPGASGPGQQGPYGPGASAAAAAAAGPGQYVLIGPGQQGPSASAAAAAAAGSYGSGPGQYGPYGPGQSGPGSGQQGQGPYGPGASAAAAAAAGSYGPGQQVLIGPYGPGPSAAAAAAAGPGSGQYGPGASGQNGPGSGQYGPGQQGPGPSAAAAAAAGPGSGQQGPGASVLI

SEQ ID NO: 24 - protein, 630 aa, Artificial Sequence
  PRT666
MHHHHHHSSGSSGPGQQGPYGPGASAAAAAAAGSNGPGSGQQGPGQSGQYGPGQQGPGQQGPGSSAAAAAAAGPGQYVLIGPGQQVLIGPSASAAAAAAAGPGSGQQGPGASGQYGPGQQGPGQQGPGSSAAAAAAAGSYGSVLIGPGQQVLIGPYGSAAAAAAAGPGSGQYGQGPYGPGASGPGQYGPGQQGPSASAAAAAAAGSGQQVLIGPGQYVLIGPYASAAAAAAAGSYGSGPGQQGPYGPGQSGSGQQGPGQQGPYASAAAAAAAGPGQQVLIGPYVLIGPGSSAAAAAAAGSYGYGPGQQGPYGPGASGQNGPGSGQYGPGQQGPGPSAAAAAAAGPGQQVLIGPYVLIGPGASAAAAAAAGSYGPGQQGPGQYGPGSSGPGQQGPYGPGSSAAAAAAAGSYGPGQQVLIGPYVLIGPGPSAAAAAAAGSYQQGPGQQGPYGPGASGPGQQGPYGPGASAAAAAAAGPGQYVLIGPGQQVLIGPSASAAAAAAAGSYGSGPGQYGPYGPGQSGPGSGQQGQGPYGPGASAAAAAAAGSYGPGQQVLIGPYVLIGPGPSAAAAAAAGPGSGQYGPGASGQNGPGSGQYGPGQQGPGPSAAAAAAAGPGSGQQVLIGPGASVLI

SEQ ID NO: 25 - protein, 593 aa, Artificial Sequence
  Met-PRT888
MGSSGPGVLGPYGPGASAAAAAGQNGPGSGVLGPGQSGQYGPGVLGPGVLGPGSSAAAAAGPGQYGPGVLGPSASAAAAAGPGSGVLGPGASGQYGPGVLGPGVLGPGSSAAAAAGQYGSGPGVLGPYGSAAAAAGPGSGQYGQGPYGPGASGPGQYGPGVLGPSASAAAAAGSGVLGPGQYGPYASAAAAAGQYGSGPGVLGPYGPGQSGSGVLGPGVLGPYASAAAAAGPGVLGPYGPGSSAAAAAGQYGYGPGVLGPYGPGASGQNGPGSGQYGPGVLGPGQSAAAAAGPGVLGPYGPGASAAAAAGQYGPGVLGPGQYGPGSSGPGVLGPYGPGSSAAAAAGQYGPGVLGPYGPGQSAAAAAGQYVLGPGVLGPYGPGASGPGVLGPYGPGASAAAAAGPGQYGPGVLGPSASAAAAAGQYGSGPGQYGPYGPGQSGPGSGVLGQGPYGPGASAAAAAGQYGPGVLGPYGPGQSAAAAAGPGSGQYGPGASGQNGPGSGQYGPGVLGPGQSAAAAAGQYVLGPGVLGPYGPGASAAAAAGQYGSGPGVLGPYGPGQSGSGVLGPGVLGPYASAAAAAGPGSGVLGPGAS

SEQ ID NO: 26 - protein, 590 aa, Artificial Sequence
  Met-PRT965
MGPGTSGPYGPGASAAAAAGANGPGSGTSGPGASGAYGPGTSGPGTSGPGSSAAAAAGPGAYGPGTSGPSASAAAAAGPGSGTSGPGASGAYGPGTSGPGTSGPGSSAAAAAGAYGSGPGTSGPYGSAAAAAGPGSGAYGAGPYGPGASGPGAYGPGTSGPSASAAAAAGSGTSGPGAYGPYASAAAAAGAYGSGPGTSGPYGPGASGSGTSGPGTSGPYASAAAAAGPGTSGPYGPGSSAAAAAGAYGYGPGTSGPYGPGASGANGPGSGAYGPGTSGPGASAAAAAGPGTSGPYGPGASAAAAAGAYGPGTSGPGAYGPGSSGPGTSGPYGPGSSAAAAAGAYGPGTSGPYGPGASAAAAAGAYTSGPGTSGPYGPGASGPGTSGPYGPGASAAAAAGPGAYGPGTSGPSASAAAAAGAYGSGPGAYGPYGPGASGPGSGTSGAGPYGPGASAAAAAGAYGPGTSGPYGPGASAAAAAGPGSGAYGPGASGANGPGSGAYGPGTSGPGASAAAAAGAYTSGPGTSGPYGPGASAAAAAGAYGSGPGTSGPYGPGASGSGTSGPGTSGPYASAAAAAGPGSGTSGPGAS

SEQ ID NO: 27 - protein, 593 aa, Artificial Sequence
  Met-PRT889
MGSSGPGVLGPYGPGASAAAAAGINGPGSGVLGPGISGIYGPGVLGPGVLGPGSSAAAAAGPGIYGPGVLGPSASAAAAAGPGSGVLGPGASGIYGPGVLGPGVLGPGSSAAAAAGIYGSGPGVLGPYGSAAAAAGPGSGIYGIGPYGPGASGPGIYGPGVLGPSASAAAAAGSGVLGPGIYGPYASAAAAAGIYGSGPGVLGPYGPGISGSGVLGPGVLGPYASAAAAAGPGVLGPYGPGSSAAAAAGIYGYGPGVLGPYGPGASGINGPGSGIYGPGVLGPGISAAAAAGPGVLGPYGPGASAAAAAGIYGPGVLGPGIYGPGSSGPGVLGPYGPGSSAAAAAGIYGPGVLGPYGPGISAAAAAGIYVLGPGVLGPYGPGASGPGVLGPYGPGASAAAAAGPGIYGPGVLGPSASAAAAAGIYGSGPGIYGPYGPGISGPGSGVLGIGPYGPGASAAAAAGIYGPGVLGPYGPGISAAAAAGPGSGIYGPGASGINGPGSGIYGPGVLGPGISAAAAAGIYVLGPGVLGPYGPGASAAAAAGIYGSGPGVLGPYGPGISGSGVLGPGVLGPYASAAAAAGPGSGVLGPGAS

SEQ ID NO: 28 - protein, 590 aa, Artificial Sequence
  Met-PRT916
MGPGVIGPYGPGASAAAAAGLNGPGSGVIGPGLSGLYGPGVIGPGVIGPGSSAAAAAGPGLYGPGVIGPSASAAAAAGPGSGVIGPGASGLYGPGVIGPGVIGPGSSAAAAAGLYGSGPGVIGPYGSAAAAAGPGSGLYGLGPYGPGASGPGLYGPGVIGPSASAAAAAGSGVIGPGLYGPYASAAAAAGLYGSGPGVIGPYGPGLSGSGVIGPGVIGPYASAAAAAGPGVIGPYGPGSSAAAAAGLYGYGPGVIGPYGPGASGLNGPGSGLYGPGVIGPGLSAAAAAGPGVIGPYGPGASAAAAAGLYGPGVIGPGLYGPGSSGPGVIGPYGPGSSAAAAAGLYGPGVIGPYGPGLSAAAAAGLYVIGPGVIGPYGPGASGPGVIGPYGPGASAAAAAGPGLYGPGVIGPSASAAAAAGLYGSGPGLYGPYGPGLSGPGSGVIGLGPYGPGASAAAAAGLYGPGVIGPYGPGLSAAAAAGPGSGLYGPGASGLNGPGSGLYGPGVIGPGLSAAAAAGLYVIGPGVIGPYGPGASAAAAAGLYGSGPGVIGPYGPGLSGSGVIGPGVIGPYASAAAAAGPGSGVIGPGAS

SEQ ID NO: 29 - protein, 590 aa, Artificial Sequence
  Met-PRT918
MGPGVFGPYGPGASAAAAAGINGPGSGVFGPGISGIYGPGVFGPGVFGPGSSAAAAAGPGIYGPGVFGPSASAAAAAGPGSGVFGPGASGIYGPGVFGPGVFGPGSSAAAAAGIYGSGPGVFGPYGSAAAAAGPGSGIYGIGPYGPGASGPGIYGPGVFGPSASAAAAAGSGVFGPGIYGPYASAAAAAGIYGSGPGVFGPYGPGISGSGVFGPGVFGPYASAAAAAGPGVFGPYGPGSSAAAAAGIYGYGPGVFGPYGPGASGINGPGSGIYGPGVFGPGISAAAAAGPGVFGPYGPGASAAAAAGIYGPGVFGPGIYGPGSSGPGVFGPYGPGSSAAAAAGIYGPGVFGPYGPGISAAAAAGIYVFGPGVFGPYGPGASGPGVFGPYGPGASAAAAAGPGIYGPGVFGPSASAAAAAGIYGSGPGIYGPYGPGISGPGSGVFGIGPYGPGASAAAAAGIYGPGVFGPYGPGISAAAAAGPGSGIYGPGASGINGPGSGIYGPGVFGPGISAAAAAGIYVFGPGVFGPYGPGASAAAAAGIYGSGPGVFGPYGPGISGSGVFGPGVFGPYASAAAAAGPGSGVFGPGAS

SEQ ID NO: 30 - protein, 565 aa, Artificial Sequence
  Met-PRT699
MGPGVLGPYGPGASAAAAAAAGSNGPGSGVLGPGQSGQYGPGVLGPGVLGPGSSAAAAAAAGPGQYGPGVLGPSASAAAAAAAGPGSGVLGPGASGQYGPGVLGPGVLGPGSSAAAAAAAGSYGSGPGVLGPYGSAAAAAAAGPGSGQYGQGPYGPGASGPGQYGPGVLGPSASAAAAAAAGSGVLGPGQYGPYASAAAAAAAGSYGSGPGVLGPYGPGQSGSGVLGPGVLGPYASAAAAAAAGPGVLGPYGPGSSAAAAAAAGSYGYGPGVLGPYGPGASGQNGPGSGQYGPGVLGPGPSAAAAAAAGPGVLGPYGPGASAAAAAAAGSYGPGVLGPGQYGPGSSGPGVLGPYGPGSSAAAAAAAGSYGPGVLGPYGPGPSAAAAAAAGSYVLGPGVLGPYGPGASGPGVLGPYGPGASAAAAAAAGPGQYGPGVLGPSASAAAAAAAGSYGSGPGQYGPYGPGQSGPGSGVLGQGPYGPGASAAAAAAAGSYGPGVLGPYGPGPSAAAAAAAGPGSGQYGPGASGQNGPGSGQYGPGVLGPGPSAAAAAAAGPGSGVLGPGAS

SEQ ID NO: 31 - protein, 565 aa, Artificial Sequence
  Met-PRT698
MGPGVLGPYGPGASAAAAAAAGSNGPGSGVLGPGISGIYGPGVLGPGVLGPGSSAAAAAAAGPGIYGPGVLGPSASAAAAAAAGPGSGVLGPGASGIYGPGVLGPGVLGPGSSAAAAAAAGSYGSGPGVLGPYGSAAAAAAAGPGSGIYGIGPYGPGASGPGIYGPGVLGPSASAAAAAAAGSGVLGPGIYGPYASAAAAAAAGSYGSGPGVLGPYGPGISGSGVLGPGVLGPYASAAAAAAAGPGVLGPYGPGSSAAAAAAAGSYGYGPGVLGPYGPGASGINGPGSGIYGPGVLGPGPSAAAAAAAGPGVLGPYGPGASAAAAAAAGSYGPGVLGPGIYGPGSSGPGVLGPYGPGSSAAAAAAAGSYGPGVLGPYGPGPSAAAAAAAGSYVLGPGVLGPYGPGASGPGVLGPYGPGASAAAAAAAGPGIYGPGVLGPSASAAAAAAAGSYGSGPGIYGPYGPGISGPGSGVLGIGPYGPGASAAAAAAAGSYGPGVLGPYGPGPSAAAAAAAGPGSGIYGPGASGINGPGSGIYGPGVLGPGPSAAAAAAAGPGSGVLGPGAS

SEQ ID NO: 32 - protein, 1179 aa, Artificial Sequence
  Met-PRT966
MGPGVFGPYGPGASAAAAAGINGPGSGVFGPGISGIYGPGVFGPGVFGPGSSAAAAAGPGIYGPGVFGPSASAAAAAGPGSGVFGPGASGIYGPGVFGPGVFGPGSSAAAAAGIYGSGPGVFGPYGSAAAAAGPGSGIYGIGPYGPGASGPGIYGPGVFGPSASAAAAAGSGVFGPGIYGPYASAAAAAGIYGSGPGVFGPYGPGISGSGVFGPGVFGPYASAAAAAGPGVFGPYGPGSSAAAAAGIYGYGPGVFGPYGPGASGINGPGSGIYGPGVFGPGISAAAAAGPGVFGPYGPGASAAAAAGIYGPGVFGPGIYGPGSSGPGVFGPYGPGSSAAAAAGIYGPGVFGPYGPGISAAAAAGIYVFGPGVFGPYGPGASGPGVFGPYGPGASAAAAAGPGIYGPGVFGPSASAAAAAGIYGSGPGIYGPYGPGISGPGSGVFGIGPYGPGASAAAAAGIYGPGVFGPYGPGISAAAAAGPGSGIYGPGASGINGPGSGIYGPGVFGPGISAAAAAGIYVFGPGVFGPYGPGASAAAAAGIYGSGPGVFGPYGPGISGSGVFGPGVFGPYASAAAAAGPGSGVFGPGASGPGVFGPYGPGASAAAAAGINGPGSGVFGPGISGIYGPGVFGPGVFGPGSSAAAAAGPGIYGPGVFGPSASAAAAAGPGSGVFGPGASGIYGPGVFGPGVFGPGSSAAAAAGIYGSGPGVFGPYGSAAAAAGPGSGIYGIGPYGPGASGPGIYGPGVFGPSASAAAAAGSGVFGPGIYGPYASAAAAAGIYGSGPGVFGPYGPGISGSGVFGPGVFGPYASAAAAAGPGVFGPYGPGSSAAAAAGIYGYGPGVFGPYGPGASGINGPGSGIYGPGVFGPGISAAAAAGPGVFGPYGPGASAAAAAGIYGPGVFGPGIYGPGSSGPGVFGPYGPGSSAAAAAGIYGPGVFGPYGPGISAAAAAGIYVFGPGVFGPYGPGASGPGVFGPYGPGASAAAAAGPGIYGPGVFGPSASAAAAAGIYGSGPGIYGPYGPGISGPGSGVFGIGPYGPGASAAAAAGIYGPGVFGPYGPGISAAAAAGPGSGIYGPGASGINGPGSGIYGPGVFGPGISAAAAAGIYVFGPGVFGPYGPGASAAAAAGIYGSGPGVFGPYGPGISGSGVFGPGVFGPYASAAAAAGPGSGVFGPGAS

SEQ ID NO: 33 - protein, 601 aa, Artificial Sequence
  PRT888
MHHHHHHSSGSSGPGVLGPYGPGASAAAAAGQNGPGSGVLGPGQSGQYGPGVLGPGVLGPGSSAAAAAGPGQYGPGVLGPSASAAAAAGPGSGVLGPGASGQYGPGVLGPGVLGPGSSAAAAAGQYGSGPGVLGPYGSAAAAAGPGSGQYGQGPYGPGASGPGQYGPGVLGPSASAAAAAGSGVLGPGQYGPYASAAAAAGQYGSGPGVLGPYGPGQSGSGVLGPGVLGPYASAAAAAGPGVLGPYGPGSSAAAAAGQYGYGPGVLGPYGPGASGQNGPGSGQYGPGVLGPGQSAAAAAGPGVLGPYGPGASAAAAAGQYGPGVLGPGQYGPGSSGPGVLGPYGPGSSAAAAAGQYGPGVLGPYGPGQSAAAAAGQYVLGPGVLGPYGPGASGPGVLGPYGPGASAAAAAGPGQYGPGVLGPSASAAAAAGQYGSGPGQYGPYGPGQSGPGSGVLGQGPYGPGASAAAAAGQYGPGVLGPYGPGQSAAAAAGPGSGQYGPGASGQNGPGSGQYGPGVLGPGQSAAAAAGQYVLGPGVLGPYGPGASAAAAAGQYGSGPGVLGPYGPGQSGSGVLGPGVLGPYASAAAAAGPGSGVLGPGAS

SEQ ID NO: 34 - protein, 601 aa, Artificial Sequence
  PRT965
MHHHHHHSSGSSGPGTSGPYGPGASAAAAAGANGPGSGTSGPGASGAYGPGTSGPGTSGPGSSAAAAAGPGAYGPGTSGPSASAAAAAGPGSGTSGPGASGAYGPGTSGPGTSGPGSSAAAAAGAYGSGPGTSGPYGSAAAAAGPGSGAYGAGPYGPGASGPGAYGPGTSGPSASAAAAAGSGTSGPGAYGPYASAAAAAGAYGSGPGTSGPYGPGASGSGTSGPGTSGPYASAAAAAGPGTSGPYGPGSSAAAAAGAYGYGPGTSGPYGPGASGANGPGSGAYGPGTSGPGASAAAAAGPGTSGPYGPGASAAAAAGAYGPGTSGPGAYGPGSSGPGTSGPYGPGSSAAAAAGAYGPGTSGPYGPGASAAAAAGAYTSGPGTSGPYGPGASGPGTSGPYGPGASAAAAAGPGAYGPGTSGPSASAAAAAGAYGSGPGAYGPYGPGASGPGSGTSGAGPYGPGASAAAAAGAYGPGTSGPYGPGASAAAAAGPGSGAYGPGASGANGPGSGAYGPGTSGPGASAAAAAGAYTSGPGTSGPYGPGASAAAAAGAYGSGPGTSGPYGPGASGSGTSGPGTSGPYASAAAAAGPGSGTSGPGAS

SEQ ID NO: 35 - protein, 601 aa, Artificial Sequence
  PRT889
MHHHHHHSSGSSGPGVLGPYGPGASAAAAAGINGPGSGVLGPGISGIYGPGVLGPGVLGPGSSAAAAAGPGIYGPGVLGPSASAAAAAGPGSGVLGPGASGIYGPGVLGPGVLGPGSSAAAAAGIYGSGPGVLGPYGSAAAAAGPGSGIYGIGPYGPGASGPGIYGPGVLGPSASAAAAAGSGVLGPGIYGPYASAAAAAGIYGSGPGVLGPYGPGISGSGVLGPGVLGPYASAAAAAGPGVLGPYGPGSSAAAAAGIYGYGPGVLGPYGPGASGINGPGSGIYGPGVLGPGISAAAAAGPGVLGPYGPGASAAAAAGIYGPGVLGPGIYGPGSSGPGVLGPYGPGSSAAAAAGIYGPGVLGPYGPGISAAAAAGIYVLGPGVLGPYGPGASGPGVLGPYGPGASAAAAAGPGIYGPGVLGPSASAAAAAGIYGSGPGIYGPYGPGISGPGSGVLGIGPYGPGASAAAAAGIYGPGVLGPYGPGISAAAAAGPGSGIYGPGASGINGPGSGIYGPGVLGPGISAAAAAGIYVLGPGVLGPYGPGASAAAAAGIYGSGPGVLGPYGPGISGSGVLGPGVLGPYASAAAAAGPGSGVLGPGAS

SEQ ID NO: 36 - protein, 601 aa, Artificial Sequence
  PRT916
MHHHHHHSSGSSGPGVIGPYGPGASAAAAAGLNGPGSGVIGPGLSGLYGPGVIGPGVIGPGSSAAAAAGPGLYGPGVIGPSASAAAAAGPGSGVIGPGASGLYGPGVIGPGVIGPGSSAAAAAGLYGSGPGVIGPYGSAAAAAGPGSGLYGLGPYGPGASGPGLYGPGVIGPSASAAAAAGSGVIGPGLYGPYASAAAAAGLYGSGPGVIGPYGPGLSGSGVIGPGVIGPYASAAAAAGPGVIGPYGPGSSAAAAAGLYGYGPGVIGPYGPGASGLNGPGSGLYGPGVIGPGLSAAAAAGPGVIGPYGPGASAAAAAGLYGPGVIGPGLYGPGSSGPGVIGPYGPGSSAAAAAGLYGPGVIGPYGPGLSAAAAAGLYVIGPGVIGPYGPGASGPGVIGPYGPGASAAAAAGPGLYGPGVIGPSASAAAAAGLYGSGPGLYGPYGPGLSGPGSGVIGLGPYGPGASAAAAAGLYGPGVIGPYGPGLSAAAAAGPGSGLYGPGASGLNGPGSGLYGPGVIGPGLSAAAAAGLYVIGPGVIGPYGPGASAAAAAGLYGSGPGVIGPYGPGLSGSGVIGPGVIGPYASAAAAAGPGSGVIGPGAS

SEQ ID NO: 37 - protein, 601 aa, Artificial Sequence
  PRT918
MHHHHHHSSGSSGPGVFGPYGPGASAAAAAGINGPGSGVFGPGISGIYGPGVFGPGVFGPGSSAAAAAGPGIYGPGVFGPSASAAAAAGPGSGVFGPGASGIYGPGVFGPGVFGPGSSAAAAAGIYGSGPGVFGPYGSAAAAAGPGSGIYGIGPYGPGASGPGIYGPGVFGPSASAAAAAGSGVFGPGIYGPYASAAAAAGIYGSGPGVFGPYGPGISGSGVFGPGVFGPYASAAAAAGPGVFGPYGPGSSAAAAAGIYGYGPGVFGPYGPGASGINGPGSGIYGPGVFGPGISAAAAAGPGVFGPYGPGASAAAAAGIYGPGVFGPGIYGPGSSGPGVFGPYGPGSSAAAAAGIYGPGVFGPYGPGISAAAAAGIYVFGPGVFGPYGPGASGPGVFGPYGPGASAAAAAGPGIYGPGVFGPSASAAAAAGIYGSGPGIYGPYGPGISGPGSGVFGIGPYGPGASAAAAAGIYGPGVFGPYGPGISAAAAAGPGSGIYGPGASGINGPGSGIYGPGVFGPGISAAAAAGIYVFGPGVFGPYGPGASAAAAAGIYGSGPGVFGPYGPGISGSGVFGPGVFGPYASAAAAAGPGSGVFGPGAS

SEQ ID NO: 38 - protein, 576 aa, Artificial Sequence
  PRT699
MHHHHHHSSGSSGPGVLGPYGPGASAAAAAAAGSNGPGSGVLGPGQSGQYGPGVLGPGVLGPGSSAAAAAAAGPGQYGPGVLGPSASAAAAAAAGPGSGVLGPGASGQYGPGVLGPGVLGPGSSAAAAAAAGSYGSGPGVLGPYGSAAAAAAAGPGSGQYGQGPYGPGASGPGQYGPGVLGPSASAAAAAAAGSGVLGPGQYGPYASAAAAAAAGSYGSGPGVLGPYGPGQSGSGVLGPGVLGPYASAAAAAAAGPGVLGPYGPGSSAAAAAAAGSYGYGPGVLGPYGPGASGQNGPGSGQYGPGVLGPGPSAAAAAAAGPGVLGPYGPGASAAAAAAAGSYGPGVLGPGQYGPGSSGPGVLGPYGPGSSAAAAAAAGSYGPGVLGPYGPGPSAAAAAAAGSYVLGPGVLGPYGPGASGPGVLGPYGPGASAAAAAAAGPGQYGPGVLGPSASAAAAAAAGSYGSGPGQYGPYGPGQSGPGSGVLGQGPYGPGASAAAAAAAGSYGPGVLGPYGPGPSAAAAAAAGPGSGQYGPGASGQNGPGSGQYGPGVLGPGPSAAAAAAAGPGSGVLGPGAS

SEQ ID NO: 39 - protein, 576 aa, Artificial Sequence
  PRT698
MHHHHHHSSGSSGPGVLGPYGPGASAAAAAAAGSNGPGSGVLGPGISGIYGPGVLGPGVLGPGSSAAAAAAAGPGIYGPGVLGPSASAAAAAAAGPGSGVLGPGASGIYGPGVLGPGVLGPGSSAAAAAAAGSYGSGPGVLGPYGSAAAAAAAGPGSGIYGIGPYGPGASGPGIYGPGVLGPSASAAAAAAAGSGVLGPGIYGPYASAAAAAAAGSYGSGPGVLGPYGPGISGSGVLGPGVLGPYASAAAAAAAGPGVLGPYGPGSSAAAAAAAGSYGYGPGVLGPYGPGASGINGPGSGIYGPGVLGPGPSAAAAAAAGPGVLGPYGPGASAAAAAAAGSYGPGVLGPGIYGPGSSGPGVLGPYGPGSSAAAAAAAGSYGPGVLGPYGPGPSAAAAAAAGSYVLGPGVLGPYGPGASGPGVLGPYGPGASAAAAAAAGPGIYGPGVLGPSASAAAAAAAGSYGSGPGIYGPYGPGISGPGSGVLGIGPYGPGASAAAAAAAGSYGPGVLGPYGPGPSAAAAAAAGPGSGIYGPGASGINGPGSGIYGPGVLGPGPSAAAAAAAGPGSGVLGPGAS

SEQ ID NO: 40 - protein, 1190 aa, Artificial Sequence
  PRT966
MHHHHHHSSGSSGPGVFGPYGPGASAAAAAGINGPGSGVFGPGISGIYGPGVFGPGVFGPGSSAAAAAGPGIYGPGVFGPSASAAAAAGPGSGVFGPGASGIYGPGVFGPGVFGPGSSAAAAAGIYGSGPGVFGPYGSAAAAAGPGSGIYGIGPYGPGASGPGIYGPGVFGPSASAAAAAGSGVFGPGIYGPYASAAAAAGIYGSGPGVFGPYGPGISGSGVFGPGVFGPYASAAAAAGPGVFGPYGPGSSAAAAAGIYGYGPGVFGPYGPGASGINGPGSGIYGPGVFGPGISAAAAAGPGVFGPYGPGASAAAAAGIYGPGVFGPGIYGPGSSGPGVFGPYGPGSSAAAAAGIYGPGVFGPYGPGISAAAAAGIYVFGPGVFGPYGPGASGPGVFGPYGPGASAAAAAGPGIYGPGVFGPSASAAAAAGIYGSGPGIYGPYGPGISGPGSGVFGIGPYGPGASAAAAAGIYGPGVFGPYGPGISAAAAAGPGSGIYGPGASGINGPGSGIYGPGVFGPGISAAAAAGIYVFGPGVFGPYGPGASAAAAAGIYGSGPGVFGPYGPGISGSGVFGPGVFGPYASAAAAAGPGSGVFGPGASGPGVFGPYGPGASAAAAAGINGPGSGVFGPGISGIYGPGVFGPGVFGPGSSAAAAAGPGIYGPGVFGPSASAAAAAGPGSGVFGPGASGIYGPGVFGPGVFGPGSSAAAAAGIYGSGPGVFGPYGSAAAAAGPGSGIYGIGPYGPGASGPGIYGPGVFGPSASAAAAAGSGVFGPGIYGPYASAAAAAGIYGSGPGVFGPYGPGISGSGVFGPGVFGPYASAAAAAGPGVFGPYGPGSSAAAAAGIYGYGPGVFGPYGPGASGINGPGSGIYGPGVFGPGISAAAAAGPGVFGPYGPGASAAAAAGIYGPGVFGPGIYGPGSSGPGVFGPYGPGSSAAAAAGIYGPGVFGPYGPGISAAAAAGIYVFGPGVFGPYGPGASGPGVFGPYGPGASAAAAAGPGIYGPGVFGPSASAAAAAGIYGSGPGIYGPYGPGISGPGSGVFGIGPYGPGASAAAAAGIYGPGVFGPYGPGISAAAAAGPGSGIYGPGASGINGPGSGIYGPGVFGPGISAAAAAGIYVFGPGVFGPYGPGASAAAAAGIYGSGPGVFGPYGPGISGSGVFGPGVFGPYASAAAAAGPGSGVFGPGAS

SEQ ID NO: 41 - protein, 590 aa, Artificial Sequence
  Met_PRT917
MGPGLIGPYGPGASAAAAAGVNGPGSGLIGPGVSGVYGPGLIGPGLIGPGSSAAAAAGPGVYGPGLIGPSASAAAAAGPGSGLIGPGASGVYGPGLIGPGLIGPGSSAAAAAGVYGSGPGLIGPYGSAAAAAGPGSGVYGVGPYGPGASGPGVYGPGLIGPSASAAAAAGSGLIGPGVYGPYASAAAAAGVYGSGPGLIGPYGPGVSGSGLIGPGLIGPYASAAAAAGPGLIGPYGPGSSAAAAAGVYGYGPGLIGPYGPGASGVNGPGSGVYGPGLIGPGVSAAAAAGPGLIGPYGPGASAAAAAGVYGPGLIGPGVYGPGSSGPGLIGPYGPGSSAAAAAGVYGPGLIGPYGPGVSAAAAAGVYLIGPGLIGPYGPGASGPGLIGPYGPGASAAAAAGPGVYGPGLIGPSASAAAAAGVYGSGPGVYGPYGPGVSGPGSGLIGVGPYGPGASAAAAAGVYGPGLIGPYGPGVSAAAAAGPGSGVYGPGASGVNGPGSGVYGPGLIGPGVSAAAAAGVYLIGPGLIGPYGPGASAAAAAGVYGSGPGLIGPYGPGVSGSGLIGPGLIGPYASAAAAAGPGSGLIGPGAS

SEQ ID NO: 42 - protein, 587 aa, Artificial Sequence
  Met_PRT1028
MGPGIFGPYGPGASAAAAAGTGPGSGIFGPGTSGTYGPGIFGPGIFGPGSSAAAAAGPGTYGPGIFGPSASAAAAAGPGSGIFGPGASGTYGPGIFGPGIFGPGSSAAAAAGTYGSGPGIFGPYGSAAAAAGPGSGTYGTGPYGPGASGPGTYGPGIFGPSASAAAAAGSGIFGPGTYGPYASAAAAAGTYGSGPGIFGPYGPGTSGSGIFGPGIFGPYASAAAAAGPGIFGPYGPGSSAAAAAGTYGYGPGIFGPYGPGASGTGPGSGTYGPGIFGPGTSAAAAAGPGIFGPYGPGASAAAAAGTYGPGIFGPGTYGPGSSGPGIFGPYGPGSSAAAAAGTYGPGIFGPYGPGTSAAAAAGTYIFGPGIFGPYGPGASGPGIFGPYGPGASAAAAAGPGTYGPGIFGPSASAAAAAGTYGSGPGTYGPYGPGTSGPGSGIFGTGPYGPGASAAAAAGTYGPGIFGPYGPGTSAAAAAGPGSGTYGPGASGTGPGSGTYGPGIFGPGTSAAAAAGTYIFGPGIFGPYGPGASAAAAAGTYGSGPGIFGPYGPGTSGSGIFGPGIFGPYASAAAAAGPGSGIFGPGAS

SEQ ID NO: 43 - protein, 601 aa, Artificial Sequence
  PRT917
MHHHHHHSSGSSGPGLIGPYGPGASAAAAAGVNGPGSGLIGPGVSGVYGPGLIGPGLIGPGSSAAAAAGPGVYGPGLIGPSASAAAAAGPGSGLIGPGASGVYGPGLIGPGLIGPGSSAAAAAGVYGSGPGLIGPYGSAAAAAGPGSGVYGVGPYGPGASGPGVYGPGLIGPSASAAAAAGSGLIGPGVYGPYASAAAAAGVYGSGPGLIGPYGPGVSGSGLIGPGLIGPYASAAAAAGPGLIGPYGPGSSAAAAAGVYGYGPGLIGPYGPGASGVNGPGSGVYGPGLIGPGVSAAAAAGPGLIGPYGPGASAAAAAGVYGPGLIGPGVYGPGSSGPGLIGPYGPGSSAAAAAGVYGPGLIGPYGPGVSAAAAAGVYLIGPGLIGPYGPGASGPGLIGPYGPGASAAAAAGPGVYGPGLIGPSASAAAAAGVYGSGPGVYGPYGPGVSGPGSGLIGVGPYGPGASAAAAAGVYGPGLIGPYGPGVSAAAAAGPGSGVYGPGASGVNGPGSGVYGPGLIGPGVSAAAAAGVYLIGPGLIGPYGPGASAAAAAGVYGSGPGLIGPYGPGVSGSGLIGPGLIGPYASAAAAAGPGSGLIGPGAS

SEQ ID NO: 44 - protein, 598 aa, Artificial Sequence
  PRT1028
MHHHHHHSSGSSGPGIFGPYGPGASAAAAAGTGPGSGIFGPGTSGTYGPGIFGPGIFGPGSSAAAAAGPGTYGPGIFGPSASAAAAAGPGSGIFGPGASGTYGPGIFGPGIFGPGSSAAAAAGTYGSGPGIFGPYGSAAAAAGPGSGTYGTGPYGPGASGPGTYGPGIFGPSASAAAAAGSGIFGPGTYGPYASAAAAAGTYGSGPGIFGPYGPGTSGSGIFGPGIFGPYASAAAAAGPGIFGPYGPGSSAAAAAGTYGYGPGIFGPYGPGASGTGPGSGTYGPGIFGPGTSAAAAAGPGIFGPYGPGASAAAAAGTYGPGIFGPGTYGPGSSGPGIFGPYGPGSSAAAAAGTYGPGIFGPYGPGTSAAAAAGTYIFGPGIFGPYGPGASGPGIFGPYGPGASAAAAAGPGTYGPGIFGPSASAAAAAGTYGSGPGTYGPYGPGTSGPGSGIFGTGPYGPGASAAAAAGTYGPGIFGPYGPGTSAAAAAGPGSGTYGPGASGTGPGSGTYGPGIFGPGTSAAAAAGTYIFGPGIFGPYGPGASAAAAAGTYGSGPGIFGPYGPGTSGSGIFGPGIFGPYASAAAAAGPGSGIFGPGAS

SEQ ID NO: 45 - protein, 252 aa, Artificial Sequence
  Collagen-type4-Kai
MHHHHHHSSGSSKDGVPGFPGSEGVKGNRGFPGLMGEDGIKGQKGDIGPPGFRGPTEYYDTYQEKGDEGTPGPPGPRGARGPQGPSGPPGVPGSPGSSRPGLRGAPGWPGLKGSKGERGRPGKDAMGTPGSPGCAGSPGLPGSPGPPGPPGDIVFRKGPPGDHGLPGYLGSPGIPGVDGPKGEPGLLCTQCPYIPGPPGLPGLPGLHGVKGIPGRQGAAGLKGSPGSPGNTGLPGFPGFPGAQGDPGLKGEK

SEQ ID NO: 46 - protein, 310 aa, Artificial Sequence
  Resilin-Kai
MHHHHHHPEPPVNSYLPPSDSYGAPGQSGPGGRPSDSYGAPGGGNGGRPSDSYGAPGQGQGQGQGQGGYAGKPSDSYGAPGGGDGNGGRPSSSYGAPGGGNGGRPSDTYGAPGGGNGGRPSDTYGAPGGGGNGNGGRPSSSYGAPGQGQGNGNGGRPSSSYGAPGGGNGGRPSDTYGAPGGGNGGRPSDTYGAPGGGNNGGRPSSSYGAPGGGNGGRPSDTYGAPGGGNGNGSGGRPSSSYGAPGQGQGGFGGRPSDSYGAPGQNQKPSDSYGAPGSGNGNGGRPSSSYGAPGSGPGGRPSDSYGPPASG

SEQ ID NO: 47 - protein, 282 aa, Artificial Sequence
  elastin short
MHHHHHHSSGSSLGVSAGAVVPQPGAGVKPGKVPGVGLPGVYPGGVLPGARFPGVGVLPGVPTGAGVKPKAPGVGGAFAGIPGVGPFGGPQPGVPLGYPIKAPKLPGGYGLPYTTGKLPYGYGPGGVAGAAGKAGYPTGTGVGPQAAAAAAAKAAAKFGAGAAGVLPGVGGAGVPGVPGAIPGIGGIAGVGTPAAAAAAAAAAKAAKYGAAAGLVPGGPGFGPGVVGVPGAGVPGVGVPGAGIPVVPGAGIPGAAVPGVVSPEAAAKAAAKAAKYGARPGVG

SEQ ID NO: 48 - protein, 468 aa, Artificial Sequence
  type I keratin 26
MSFRLSGVSRRLCSQAGTGRLTGGRTGFRAGNVCSGLGAGSSFSGPLGSVSSKGSFSHGGGGLGSGVCTGFLENEHGLLPGNEKVTLQNLNDRLASYLDHVCTLEEANADLEQKIKGWYEKYGPGSGRQLAHDYSKYFSVTEDLKRQIISVTTCNASIVLQNENARLTADDFRLKCENELALHQSVEADINGLHRVMDELTLCTSDLEMQCEALSEELTYLKKNHQEEMKVMQGAARGNVNVEINAAPGVDLTVLLNNMRAEYEDLAEQNHEDAEAWFSEKSTSLHQQISDDAGAAMAARNELMELKRNLQTLEIELQSLLAMKHSYECSLAETESNYCHQLQQIQEQIGAMEDQLQQIRMETEGQKLEHERLLDVKIFLEKEIEMYCKLIDGEGRKSKSTCYKSEGRGPKNSENQVKDSKEEAVVKTVVGELDQLGSVLSLRVHSVEEKSSKISNITMEQRLPSKVP